European Patent Specification EP 4 004 548 B1, published January 14, 2026. Title: METHODS OF TREATING AND DIAGNOSING LUNG CANCER. Applicant: YEDA RESEARCH AND DEVELOPMENT CO. LTD. MERBL, Yifat JAVITT, Aaron KACEN, Assaf EISENBERG-LERNER, Avital SHMUELI, Merav. The sequence listing filed with the application follows.

SEQUENCE LISTING (5 sequences)

SEQ ID NO: 1 - protein, 4 aa, Artificial Sequence
  Synthetic peptide
  MISC_FEATURE (1)..(1): N-terminal succinyl conjugate
  MISC_FEATURE (4)..(4): 7-amino-4-methylcoumarin (AMC) labeled
LLVY

SEQ ID NO: 2 - protein, 3 aa, Artificial Sequence
  Synthetic peptide
  MISC_FEATURE (1)..(1): N-terminal Acetylation
  MISC_FEATURE (3)..(3): 7-amino-4-methylcoumarin (AMC) labeled
PAL

SEQ ID NO: 3 - protein, 3 aa, Artificial Sequence
  Synthetic peptide
  MISC_FEATURE (1)..(1): benzyloxycarbonyl  (Z) conjugated
  MISC_FEATURE (3)..(3): 7-amino-4-methylcoumarin (AMC) labeled
LLE

SEQ ID NO: 4 - protein, 4 aa, Artificial Sequence
  Synthetic peptide
  MISC_FEATURE (1)..(1): N-terminal Acetylation
  MISC_FEATURE (4)..(4): 7-amino-4-methylcoumarin (AMC) labeled
NPND

SEQ ID NO: 5 - protein, 3 aa, Artificial Sequence
  Synthetic peptide
  MISC_FEATURE (1)..(1): benzyloxycarbonyl  (Z)  conjugated
  MISC_FEATURE (3)..(3): betta-naphtylamide (betta-NA) conjugated
LLE